European Patent Application EP 4 803 544 A2, published September 9, 2026. Title: ANTIBODY OLIGONUCLEOTIDE CONJUGATE COMPOSITIONS AND METHODS OF INDUCING DMD EXON 44 SKIPPING. Applicant: AVIDITY BIOSCIENCES, INC. Application US PCT/US2023/017574, filed April 5, 2023. The sequence listing filed with the application follows.

SEQUENCE LISTING (134 sequences)

SEQ ID NO: 1-11 - skipped (11 entries)

SEQ ID NO: 12 - protein, 17 aa, synthetic construct
  VARIANT 6: note = N or Q
EINPIXGRSNYAZKFQG

SEQ ID NO: 13 - protein, 11 aa, synthetic construct
  VARIANT 8: note = N or S
RTSENIYXNLA

SEQ ID NO: 14 - protein, 7 aa, synthetic construct
  VARIANT 2: note = A or G
  VARIANT 7: note = D or E
AXTNLAX

SEQ ID NO: 15 - protein, 10 aa, synthetic construct
  VARIANT 10: note = May be deleted
QHFWGTPLTF

SEQ ID NO: 16 - protein, 7 aa, synthetic construct
  VARIANT 7: note = D or E
AATNLAX

SEQ ID NO: 17 - protein, 9 aa, synthetic construct
YTFTNYWMH

SEQ ID NO: 18 - protein, 17 aa, synthetic construct
EINPINGRSNYAQKFQG

SEQ ID NO: 19 - protein, 7 aa, synthetic construct
GTRAMHY

SEQ ID NO: 20 - protein, 17 aa, synthetic construct
EINPINGRSNYAEKFQG

SEQ ID NO: 21 - protein, 17 aa, synthetic construct
EINPIQGRSNYAEKFQG

SEQ ID NO: 22 - protein, 11 aa, synthetic construct
RTSENIYNNLA

SEQ ID NO: 23 - protein, 7 aa, synthetic construct
AATNLAD

SEQ ID NO: 24 - protein, 9 aa, synthetic construct
QHFWGTPLT

SEQ ID NO: 25 - protein, 7 aa, synthetic construct
AATNLAE

SEQ ID NO: 26 - protein, 10 aa, synthetic construct
QHFWGTPLTF

SEQ ID NO: 27 - protein, 11 aa, synthetic construct
RTSENIYSNLA

SEQ ID NO: 28 - protein, 7 aa, synthetic construct
AGTNLAD

SEQ ID NO: 29 - protein, 116 aa, synthetic construct
QVQLVQSGAEVKKPGASVKVSCKASGYTFTNYWMHWVRQAPGQGLEWMGEINPINGRSNYAQKFQGRVTLTVDTSISTAYMELSRLRSDDTAVYYCARGTRAMHYWGQGTLVTVSS

SEQ ID NO: 30 - protein, 116 aa, synthetic construct
QVQLVQSGAEVKKPGASVKVSCKASGYTFTNYWMHWVRQAPGQGLEWIGEINPINGRSNYAEKFQGRVTLTVDTSSSTAYMELSRLRSDDTAVYYCARGTRAMHYWGQGTLVTVSS

SEQ ID NO: 31 - protein, 116 aa, synthetic construct
QVQLVQSGAEVKKPGASVKVSCKASGYTFTNYWMHWVRQAPGQGLEWMGEINPIQGRSNYAEKFQGRVTLTVDTSSSTAYMELSSLRSEDTATYYCARGTRAMHYWGQGTLVTVSS

SEQ ID NO: 32 - protein, 116 aa, synthetic construct
QVQLVQSGAEVKKPGASVKVSCKASGYTFTNYWMHWVRQAPGQGLEWMGEINPINGRSNYAEKFQGRVTLTVDTSSSTAYMELSSLRSEDTATYYCARGTRAMHYWGQGTLVTVSS

SEQ ID NO: 33 - protein, 116 aa, synthetic construct
QVQLQQPGAELVKPGASVKLSCKASGYTFTNYWMHWVKQRPGQGLEWIGEINPINGRSNYGERFKTKATLTVDKSSSTAYMQLSSLTSEDSAVYYCARGTRAMHYWGQGTSVTVSS

SEQ ID NO: 34 - protein, 107 aa, synthetic construct
DIQMTQSPSSLSASVGDRVTITCRTSENIYNNLAWYQQKPGKSPKLLIYAATNLADGVPSRFSGSGSGTDYTLTISSLQPEDFATYYCQHFWGTPLTFGGGTKVEIK

SEQ ID NO: 35 - protein, 107 aa, synthetic construct
DIQMTQSPSSLSASVGDRVTITCRTSENIYNNLAWYQQKPGKAPKLLIYAATNLADGVPSRFSGSGSGTDYTLTISSLQPEDFATYYCQHFWGTPLTFGGGTKVEIK

SEQ ID NO: 36 - protein, 107 aa, synthetic construct
DIQMTQSPSSLSASVGDRVTITCRTSENIYNNLAWYQQKPGKAPKLLIYAATNLAEGVPSRFSGSGSGTDYTLTISSLQPEDFATYYCQHFWGTPLTFGGGTKVEIK

SEQ ID NO: 37 - protein, 107 aa, synthetic construct
DIQMTQSPSSLSASVGDRVTITCRTSENIYSNLAWYQQKPGKAPKLLIYAGTNLADGVPSRFSGSGSGTDYTLTISSLQPEDFANYYCQHFWGTPLTFGGGTKVEIK

SEQ ID NO: 38 - protein, 107 aa, synthetic construct
DIQMTQSPASLSVSVGETVTITCRTSENIYNNLAWYQQKQGKSPQLLVYAATNLADGVPSRFSGSGSGTQYSLKINSLQSEDFGNYYCQHFWGTPLTFGAGTKLELK

SEQ ID NO: 39 - protein, 445 aa, synthetic construct
QVQLVQSGAEVKKPGASVKVSCKASGYTFTNYWMHWVRQAPGQGLEWMGEINPINGRSNYAQKFQGRVTLTVDTSISTAYMELSRLRSDDTAVYYCARGTRAMHYWGQGTLVTVSSASTKGPSVFPLAPSSKSTSGGTAALGCLVKDYFPEPVTVSWNSGALTSGVHTFPAVLQSSGLYSLSSVVTVPSSSLGTQTYICNVNHKPSNTKVDKRVEPKSCDKTHTCPPCPAPELLGGPSVFLFPPKPKDTLMISRTPEVTCVVVDVSHEDPEVKFNWYVDGVEVHNAKTKPREEQYNSTYRVVSVLTVLHQDWLNGKEYKCKVSNKALPAPIEKTISKAKGQPREPQVYTLPPSREEMTKNQVSLTCLVKGFYPSDIAVEWESNGQPENNYKTTPPVLDSDGSFFLYSKLTVDKSRWQQGNVFSCSVMHEALHNHYTQKSLSLSPG

SEQ ID NO: 40 - protein, 445 aa, synthetic construct
QVQLVQSGAEVKKPGASVKVSCKASGYTFTNYWMHWVRQAPGQGLEWMGEINPINGRSNYAQKFQGRVTLTVDTSISTAYMELSRLRSDDTAVYYCARGTRAMHYWGQGTLVTVSSASTKGPSVFPLAPSSKSTSGGTAALGCLVKDYFPEPVTVSWNSGALTSGVHTFPAVLQSSGLYSLSSVVTVPSSSLGTQTYICNVNHKPSNTKVDKRVEPKSCDKTHTCPPCPAPEAAGGPSVFLFPPKPKDTLMISRTPEVTCVVVDVSHEDPEVKFNWYVDGVEVHNAKTKPREEQYNSTYRVVSVLTVLHQDWLNGKEYKCKVSNKALPAPIEKTISKAKGQPREPQVYTLPPSREEMTKNQVSLTCLVKGFYPSDIAVEWESNGQPENNYKTTPPVLDSDGSFFLYSKLTVDKSRWQQGNVFSCSVMHEALHNHYTQKSLSLSPG

SEQ ID NO: 41 - protein, 445 aa, synthetic construct
QVQLVQSGAEVKKPGASVKVSCKASGYTFTNYWMHWVRQAPGQGLEWMGEINPINGRSNYAQKFQGRVTLTVDTSISTAYMELSRLRSDDTAVYYCARGTRAMHYWGQGTLVTVSSASTKGPSVFPLAPSSKSTSGGTAALGCLVKDYFPEPVTVSWNSGALTSGVHTFPAVLQSSGLYSLSSVVTVPSSSLGTQTYICNVNHKPSNTKVDKRVEPKSCDKTHTCPPCPAPEAAGGPSVFLFPPKPKDTLMISRTPEVTCVVVDVSHEDPEVKFNWYVDGVEVHNAKTKPREEQYNSTYRVVSVLTVLHQDWLNGKEYKCGVSNKALPAPIEKTISKAKGQPREPQVYTLPPSREEMTKNQVSLTCLVKGFYPSDIAVEWESNGQPENNYKTTPPVLDSDGSFFLYSKLTVDKSRWQQGNVFSCSVMHEALHNHYTQKSLSLSPG

SEQ ID NO: 42 - protein, 445 aa, synthetic construct
QVQLVQSGAEVKKPGASVKVSCKASGYTFTNYWMHWVRQAPGQGLEWMGEINPINGRSNYAQKFQGRVTLTVDTSISTAYMELSRLRSDDTAVYYCARGTRAMHYWGQGTLVTVSSASTKGPSVFPLAPSSKSTSGGTAALGCLVKDYFPEPVTVSWNSGALTSGVHTFPAVLQSSGLYSLSSVVTVPSSSLGTQTYICNVNHKPSNTKVDKRVEPKSCDKTHTCPPCPAPEAAGGPSVFLFPPKPKDTLMISRTPEVTCVVVDVSHEDPEVKFNWYVDGVEVHNAKTKPREEQYNSTYRVVSVLTVLHQDWLNGKEYKCKVSNKARPAPIEKTISKAKGQPREPQVYTLPPSREEMTKNQVSLTCLVKGFYPSDIAVEWESNGQPENNYKTTPPVLDSDGSFFLYSKLTVDKSRWQQGNVFSCSVMHEALHNHYTQKSLSLSPG

SEQ ID NO: 43 - protein, 445 aa, synthetic construct
QVQLVQSGAEVKKPGASVKVSCKASGYTFTNYWMHWVRQAPGQGLEWMGEINPINGRSNYAQKFQGRVTLTVDTSISTAYMELSRLRSDDTAVYYCARGTRAMHYWGQGTLVTVSSASTKGPSVFPLAPSSKSTSGGTAALGCLVKDYFPEPVTVSWNSGALTSGVHTFPAVLQSSGLYSLSSVVTVPSSSLGTQTYICNVNHKPSNTKVDKRVEPKSCDKTHTCPPCPAPEAAGGPSVFLFPPKPKDTLMISRTPEVTCVVVDVSHEDPEVKFNWYVDGVEVHNAKTKPREEQYNSTYRVVSVLTVLHQDWLNGKEYKCKVSNKALGAPIEKTISKAKGQPREPQVYTLPPSREEMTKNQVSLTCLVKGFYPSDIAVEWESNGQPENNYKTTPPVLDSDGSFFLYSKLTVDKSRWQQGNVFSCSVMHEALHNHYTQKSLSLSPG

SEQ ID NO: 44 - protein, 445 aa, synthetic construct
QVQLVQSGAEVKKPGASVKVSCKASGYTFTNYWMHWVRQAPGQGLEWMGEINPINGRSNYAQKFQGRVTLTVDTSISTAYMELSRLRSDDTAVYYCARGTRAMHYWGQGTLVTVSSASTKGPSVFPLAPSSKSTSGGTAALGCLVKDYFPEPVTVSWNSGALTSGVHTFPAVLQSSGLYSLSSVVTVPSSSLGTQTYICNVNHKPSNTKVDKRVEPKSCDKTHTCPPCPAPELLGGPSVFLFPPKPKDTLMISRTPEVTCVVVAVSHEDPEVKFNWYVDGVEVHNAKTKPREEQYGSTYRVVSVLTVLHQDWLNGKEYKCKVSNKALPAPIEKTISKAKGQPREPQVYTLPPSREEMTKNQVSLTCLVKGFYPSDIAVEWESNGQPENNYKTTPPVLDSDGSFFLYSKLTVDKSRWQQGNVFSCSVMHEALHNHYTQKSLSLSPG

SEQ ID NO: 45 - protein, 445 aa, synthetic construct
QVQLVQSGAEVKKPGASVKVSCKASGYTFTNYWMHWVRQAPGQGLEWIGEINPINGRSNYAEKFQGRVTLTVDTSSSTAYMELSRLRSDDTAVYYCARGTRAMHYWGQGTLVTVSSASTKGPSVFPLAPSSKSTSGGTAALGCLVKDYFPEPVTVSWNSGALTSGVHTFPAVLQSSGLYSLSSVVTVPSSSLGTQTYICNVNHKPSNTKVDKRVEPKSCDKTHTCPPCPAPELLGGPSVFLFPPKPKDTLMISRTPEVTCVVVDVSHEDPEVKFNWYVDGVEVHNAKTKPREEQYNSTYRVVSVLTVLHQDWLNGKEYKCKVSNKALPAPIEKTISKAKGQPREPQVYTLPPSREEMTKNQVSLTCLVKGFYPSDIAVEWESNGQPENNYKTTPPVLDSDGSFFLYSKLTVDKSRWQQGNVFSCSVMHEALHNHYTQKSLSLSPG

SEQ ID NO: 46 - protein, 445 aa, synthetic construct
QVQLVQSGAEVKKPGASVKVSCKASGYTFTNYWMHWVRQAPGQGLEWIGEINPINGRSNYAEKFQGRVTLTVDTSSSTAYMELSRLRSDDTAVYYCARGTRAMHYWGQGTLVTVSSASTKGPSVFPLAPSSKSTSGGTAALGCLVKDYFPEPVTVSWNSGALTSGVHTFPAVLQSSGLYSLSSVVTVPSSSLGTQTYICNVNHKPSNTKVDKRVEPKSCDKTHTCPPCPAPEAAGGPSVFLFPPKPKDTLMISRTPEVTCVVVDVSHEDPEVKFNWYVDGVEVHNAKTKPREEQYNSTYRVVSVLTVLHQDWLNGKEYKCKVSNKALPAPIEKTISKAKGQPREPQVYTLPPSREEMTKNQVSLTCLVKGFYPSDIAVEWESNGQPENNYKTTPPVLDSDGSFFLYSKLTVDKSRWQQGNVFSCSVMHEALHNHYTQKSLSLSPG

SEQ ID NO: 47 - protein, 445 aa, synthetic construct
QVQLVQSGAEVKKPGASVKVSCKASGYTFTNYWMHWVRQAPGQGLEWIGEINPINGRSNYAEKFQGRVTLTVDTSSSTAYMELSRLRSDDTAVYYCARGTRAMHYWGQGTLVTVSSASTKGPSVFPLAPSSKSTSGGTAALGCLVKDYFPEPVTVSWNSGALTSGVHTFPAVLQSSGLYSLSSVVTVPSSSLGTQTYICNVNHKPSNTKVDKRVEPKSCDKTHTCPPCPAPEAAGGPSVFLFPPKPKDTLMISRTPEVTCVVVDVSHEDPEVKFNWYVDGVEVHNAKTKPREEQYNSTYRVVSVLTVLHQDWLNGKEYKCGVSNKALPAPIEKTISKAKGQPREPQVYTLPPSREEMTKNQVSLTCLVKGFYPSDIAVEWESNGQPENNYKTTPPVLDSDGSFFLYSKLTVDKSRWQQGNVFSCSVMHEALHNHYTQKSLSLSPG

SEQ ID NO: 48 - protein, 445 aa, synthetic construct
QVQLVQSGAEVKKPGASVKVSCKASGYTFTNYWMHWVRQAPGQGLEWIGEINPINGRSNYAEKFQGRVTLTVDTSSSTAYMELSRLRSDDTAVYYCARGTRAMHYWGQGTLVTVSSASTKGPSVFPLAPSSKSTSGGTAALGCLVKDYFPEPVTVSWNSGALTSGVHTFPAVLQSSGLYSLSSVVTVPSSSLGTQTYICNVNHKPSNTKVDKRVEPKSCDKTHTCPPCPAPEAAGGPSVFLFPPKPKDTLMISRTPEVTCVVVDVSHEDPEVKFNWYVDGVEVHNAKTKPREEQYNSTYRVVSVLTVLHQDWLNGKEYKCKVSNKARPAPIEKTISKAKGQPREPQVYTLPPSREEMTKNQVSLTCLVKGFYPSDIAVEWESNGQPENNYKTTPPVLDSDGSFFLYSKLTVDKSRWQQGNVFSCSVMHEALHNHYTQKSLSLSPG

SEQ ID NO: 49 - protein, 445 aa, synthetic construct
QVQLVQSGAEVKKPGASVKVSCKASGYTFTNYWMHWVRQAPGQGLEWIGEINPINGRSNYAEKFQGRVTLTVDTSSSTAYMELSRLRSDDTAVYYCARGTRAMHYWGQGTLVTVSSASTKGPSVFPLAPSSKSTSGGTAALGCLVKDYFPEPVTVSWNSGALTSGVHTFPAVLQSSGLYSLSSVVTVPSSSLGTQTYICNVNHKPSNTKVDKRVEPKSCDKTHTCPPCPAPEAAGGPSVFLFPPKPKDTLMISRTPEVTCVVVDVSHEDPEVKFNWYVDGVEVHNAKTKPREEQYNSTYRVVSVLTVLHQDWLNGKEYKCKVSNKALGAPIEKTISKAKGQPREPQVYTLPPSREEMTKNQVSLTCLVKGFYPSDIAVEWESNGQPENNYKTTPPVLDSDGSFFLYSKLTVDKSRWQQGNVFSCSVMHEALHNHYTQKSLSLSPG

SEQ ID NO: 50 - protein, 445 aa, synthetic construct
QVQLVQSGAEVKKPGASVKVSCKASGYTFTNYWMHWVRQAPGQGLEWIGEINPINGRSNYAEKFQGRVTLTVDTSSSTAYMELSRLRSDDTAVYYCARGTRAMHYWGQGTLVTVSSASTKGPSVFPLAPSSKSTSGGTAALGCLVKDYFPEPVTVSWNSGALTSGVHTFPAVLQSSGLYSLSSVVTVPSSSLGTQTYICNVNHKPSNTKVDKRVEPKSCDKTHTCPPCPAPELLGGPSVFLFPPKPKDTLMISRTPEVTCVVVAVSHEDPEVKFNWYVDGVEVHNAKTKPREEQYGSTYRVVSVLTVLHQDWLNGKEYKCKVSNKALPAPIEKTISKAKGQPREPQVYTLPPSREEMTKNQVSLTCLVKGFYPSDIAVEWESNGQPENNYKTTPPVLDSDGSFFLYSKLTVDKSRWQQGNVFSCSVMHEALHNHYTQKSLSLSPG

SEQ ID NO: 51 - protein, 445 aa, synthetic construct
QVQLVQSGAEVKKPGASVKVSCKASGYTFTNYWMHWVRQAPGQGLEWMGEINPIQGRSNYAEKFQGRVTLTVDTSSSTAYMELSSLRSEDTATYYCARGTRAMHYWGQGTLVTVSSASTKGPSVFPLAPSSKSTSGGTAALGCLVKDYFPEPVTVSWNSGALTSGVHTFPAVLQSSGLYSLSSVVTVPSSSLGTQTYICNVNHKPSNTKVDKRVEPKSCDKTHTCPPCPAPELLGGPSVFLFPPKPKDTLMISRTPEVTCVVVDVSHEDPEVKFNWYVDGVEVHNAKTKPREEQYNSTYRVVSVLTVLHQDWLNGKEYKCKVSNKALPAPIEKTISKAKGQPREPQVYTLPPSREEMTKNQVSLTCLVKGFYPSDIAVEWESNGQPENNYKTTPPVLDSDGSFFLYSKLTVDKSRWQQGNVFSCSVMHEALHNHYTQKSLSLSPG

SEQ ID NO: 52 - protein, 445 aa, synthetic construct
QVQLVQSGAEVKKPGASVKVSCKASGYTFTNYWMHWVRQAPGQGLEWMGEINPIQGRSNYAEKFQGRVTLTVDTSSSTAYMELSSLRSEDTATYYCARGTRAMHYWGQGTLVTVSSASTKGPSVFPLAPSSKSTSGGTAALGCLVKDYFPEPVTVSWNSGALTSGVHTFPAVLQSSGLYSLSSVVTVPSSSLGTQTYICNVNHKPSNTKVDKRVEPKSCDKTHTCPPCPAPEAAGGPSVFLFPPKPKDTLMISRTPEVTCVVVDVSHEDPEVKFNWYVDGVEVHNAKTKPREEQYNSTYRVVSVLTVLHQDWLNGKEYKCKVSNKALPAPIEKTISKAKGQPREPQVYTLPPSREEMTKNQVSLTCLVKGFYPSDIAVEWESNGQPENNYKTTPPVLDSDGSFFLYSKLTVDKSRWQQGNVFSCSVMHEALHNHYTQKSLSLSPG

SEQ ID NO: 53 - protein, 445 aa, synthetic construct
QVQLVQSGAEVKKPGASVKVSCKASGYTFTNYWMHWVRQAPGQGLEWMGEINPIQGRSNYAEKFQGRVTLTVDTSSSTAYMELSSLRSEDTATYYCARGTRAMHYWGQGTLVTVSSASTKGPSVFPLAPSSKSTSGGTAALGCLVKDYFPEPVTVSWNSGALTSGVHTFPAVLQSSGLYSLSSVVTVPSSSLGTQTYICNVNHKPSNTKVDKRVEPKSCDKTHTCPPCPAPEAAGGPSVFLFPPKPKDTLMISRTPEVTCVVVDVSHEDPEVKFNWYVDGVEVHNAKTKPREEQYNSTYRVVSVLTVLHQDWLNGKEYKCGVSNKALPAPIEKTISKAKGQPREPQVYTLPPSREEMTKNQVSLTCLVKGFYPSDIAVEWESNGQPENNYKTTPPVLDSDGSFFLYSKLTVDKSRWQQGNVFSCSVMHEALHNHYTQKSLSLSPG

SEQ ID NO: 54 - protein, 445 aa, synthetic construct
QVQLVQSGAEVKKPGASVKVSCKASGYTFTNYWMHWVRQAPGQGLEWMGEINPIQGRSNYAEKFQGRVTLTVDTSSSTAYMELSSLRSEDTATYYCARGTRAMHYWGQGTLVTVSSASTKGPSVFPLAPSSKSTSGGTAALGCLVKDYFPEPVTVSWNSGALTSGVHTFPAVLQSSGLYSLSSVVTVPSSSLGTQTYICNVNHKPSNTKVDKRVEPKSCDKTHTCPPCPAPEAAGGPSVFLFPPKPKDTLMISRTPEVTCVVVDVSHEDPEVKFNWYVDGVEVHNAKTKPREEQYNSTYRVVSVLTVLHQDWLNGKEYKCKVSNKARPAPIEKTISKAKGQPREPQVYTLPPSREEMTKNQVSLTCLVKGFYPSDIAVEWESNGQPENNYKTTPPVLDSDGSFFLYSKLTVDKSRWQQGNVFSCSVMHEALHNHYTQKSLSLSPG

SEQ ID NO: 55 - protein, 445 aa, synthetic construct
QVQLVQSGAEVKKPGASVKVSCKASGYTFTNYWMHWVRQAPGQGLEWMGEINPIQGRSNYAEKFQGRVTLTVDTSSSTAYMELSSLRSEDTATYYCARGTRAMHYWGQGTLVTVSSASTKGPSVFPLAPSSKSTSGGTAALGCLVKDYFPEPVTVSWNSGALTSGVHTFPAVLQSSGLYSLSSVVTVPSSSLGTQTYICNVNHKPSNTKVDKRVEPKSCDKTHTCPPCPAPEAAGGPSVFLFPPKPKDTLMISRTPEVTCVVVDVSHEDPEVKFNWYVDGVEVHNAKTKPREEQYNSTYRVVSVLTVLHQDWLNGKEYKCKVSNKALGAPIEKTISKAKGQPREPQVYTLPPSREEMTKNQVSLTCLVKGFYPSDIAVEWESNGQPENNYKTTPPVLDSDGSFFLYSKLTVDKSRWQQGNVFSCSVMHEALHNHYTQKSLSLSPG

SEQ ID NO: 56 - protein, 445 aa, synthetic construct
QVQLVQSGAEVKKPGASVKVSCKASGYTFTNYWMHWVRQAPGQGLEWMGEINPIQGRSNYAEKFQGRVTLTVDTSSSTAYMELSSLRSEDTATYYCARGTRAMHYWGQGTLVTVSSASTKGPSVFPLAPSSKSTSGGTAALGCLVKDYFPEPVTVSWNSGALTSGVHTFPAVLQSSGLYSLSSVVTVPSSSLGTQTYICNVNHKPSNTKVDKRVEPKSCDKTHTCPPCPAPELLGGPSVFLFPPKPKDTLMISRTPEVTCVVVAVSHEDPEVKFNWYVDGVEVHNAKTKPREEQYGSTYRVVSVLTVLHQDWLNGKEYKCKVSNKALPAPIEKTISKAKGQPREPQVYTLPPSREEMTKNQVSLTCLVKGFYPSDIAVEWESNGQPENNYKTTPPVLDSDGSFFLYSKLTVDKSRWQQGNVFSCSVMHEALHNHYTQKSLSLSPG

SEQ ID NO: 57 - protein, 445 aa, synthetic construct
QVQLVQSGAEVKKPGASVKVSCKASGYTFTNYWMHWVRQAPGQGLEWMGEINPINGRSNYAEKFQGRVTLTVDTSSSTAYMELSSLRSEDTATYYCARGTRAMHYWGQGTLVTVSSASTKGPSVFPLAPSSKSTSGGTAALGCLVKDYFPEPVTVSWNSGALTSGVHTFPAVLQSSGLYSLSSVVTVPSSSLGTQTYICNVNHKPSNTKVDKRVEPKSCDKTHTCPPCPAPELLGGPSVFLFPPKPKDTLMISRTPEVTCVVVDVSHEDPEVKFNWYVDGVEVHNAKTKPREEQYNSTYRVVSVLTVLHQDWLNGKEYKCKVSNKALPAPIEKTISKAKGQPREPQVYTLPPSREEMTKNQVSLTCLVKGFYPSDIAVEWESNGQPENNYKTTPPVLDSDGSFFLYSKLTVDKSRWQQGNVFSCSVMHEALHNHYTQKSLSLSPG

SEQ ID NO: 58 - protein, 445 aa, synthetic construct
QVQLVQSGAEVKKPGASVKVSCKASGYTFTNYWMHWVRQAPGQGLEWMGEINPINGRSNYAEKFQGRVTLTVDTSSSTAYMELSSLRSEDTATYYCARGTRAMHYWGQGTLVTVSSASTKGPSVFPLAPSSKSTSGGTAALGCLVKDYFPEPVTVSWNSGALTSGVHTFPAVLQSSGLYSLSSVVTVPSSSLGTQTYICNVNHKPSNTKVDKRVEPKSCDKTHTCPPCPAPEAAGGPSVFLFPPKPKDTLMISRTPEVTCVVVDVSHEDPEVKFNWYVDGVEVHNAKTKPREEQYNSTYRVVSVLTVLHQDWLNGKEYKCKVSNKALPAPIEKTISKAKGQPREPQVYTLPPSREEMTKNQVSLTCLVKGFYPSDIAVEWESNGQPENNYKTTPPVLDSDGSFFLYSKLTVDKSRWQQGNVFSCSVMHEALHNHYTQKSLSLSPG

SEQ ID NO: 59 - protein, 445 aa, synthetic construct
QVQLVQSGAEVKKPGASVKVSCKASGYTFTNYWMHWVRQAPGQGLEWMGEINPINGRSNYAEKFQGRVTLTVDTSSSTAYMELSSLRSEDTATYYCARGTRAMHYWGQGTLVTVSSASTKGPSVFPLAPSSKSTSGGTAALGCLVKDYFPEPVTVSWNSGALTSGVHTFPAVLQSSGLYSLSSVVTVPSSSLGTQTYICNVNHKPSNTKVDKRVEPKSCDKTHTCPPCPAPEAAGGPSVFLFPPKPKDTLMISRTPEVTCVVVDVSHEDPEVKFNWYVDGVEVHNAKTKPREEQYNSTYRVVSVLTVLHQDWLNGKEYKCGVSNKALPAPIEKTISKAKGQPREPQVYTLPPSREEMTKNQVSLTCLVKGFYPSDIAVEWESNGQPENNYKTTPPVLDSDGSFFLYSKLTVDKSRWQQGNVFSCSVMHEALHNHYTQKSLSLSPG

SEQ ID NO: 60 - protein, 445 aa, synthetic construct
QVQLVQSGAEVKKPGASVKVSCKASGYTFTNYWMHWVRQAPGQGLEWMGEINPINGRSNYAEKFQGRVTLTVDTSSSTAYMELSSLRSEDTATYYCARGTRAMHYWGQGTLVTVSSASTKGPSVFPLAPSSKSTSGGTAALGCLVKDYFPEPVTVSWNSGALTSGVHTFPAVLQSSGLYSLSSVVTVPSSSLGTQTYICNVNHKPSNTKVDKRVEPKSCDKTHTCPPCPAPEAAGGPSVFLFPPKPKDTLMISRTPEVTCVVVDVSHEDPEVKFNWYVDGVEVHNAKTKPREEQYNSTYRVVSVLTVLHQDWLNGKEYKCKVSNKARPAPIEKTISKAKGQPREPQVYTLPPSREEMTKNQVSLTCLVKGFYPSDIAVEWESNGQPENNYKTTPPVLDSDGSFFLYSKLTVDKSRWQQGNVFSCSVMHEALHNHYTQKSLSLSPG

SEQ ID NO: 61 - protein, 445 aa, synthetic construct
QVQLVQSGAEVKKPGASVKVSCKASGYTFTNYWMHWVRQAPGQGLEWMGEINPINGRSNYAEKFQGRVTLTVDTSSSTAYMELSSLRSEDTATYYCARGTRAMHYWGQGTLVTVSSASTKGPSVFPLAPSSKSTSGGTAALGCLVKDYFPEPVTVSWNSGALTSGVHTFPAVLQSSGLYSLSSVVTVPSSSLGTQTYICNVNHKPSNTKVDKRVEPKSCDKTHTCPPCPAPEAAGGPSVFLFPPKPKDTLMISRTPEVTCVVVDVSHEDPEVKFNWYVDGVEVHNAKTKPREEQYNSTYRVVSVLTVLHQDWLNGKEYKCKVSNKALGAPIEKTISKAKGQPREPQVYTLPPSREEMTKNQVSLTCLVKGFYPSDIAVEWESNGQPENNYKTTPPVLDSDGSFFLYSKLTVDKSRWQQGNVFSCSVMHEALHNHYTQKSLSLSPG

SEQ ID NO: 62 - protein, 445 aa, synthetic construct
QVQLVQSGAEVKKPGASVKVSCKASGYTFTNYWMHWVRQAPGQGLEWMGEINPINGRSNYAEKFQGRVTLTVDTSSSTAYMELSSLRSEDTATYYCARGTRAMHYWGQGTLVTVSSASTKGPSVFPLAPSSKSTSGGTAALGCLVKDYFPEPVTVSWNSGALTSGVHTFPAVLQSSGLYSLSSVVTVPSSSLGTQTYICNVNHKPSNTKVDKRVEPKSCDKTHTCPPCPAPELLGGPSVFLFPPKPKDTLMISRTPEVTCVVVAVSHEDPEVKFNWYVDGVEVHNAKTKPREEQYGSTYRVVSVLTVLHQDWLNGKEYKCKVSNKALPAPIEKTISKAKGQPREPQVYTLPPSREEMTKNQVSLTCLVKGFYPSDIAVEWESNGQPENNYKTTPPVLDSDGSFFLYSKLTVDKSRWQQGNVFSCSVMHEALHNHYTQKSLSLSPG

SEQ ID NO: 63 - protein, 214 aa, synthetic construct
DIQMTQSPSSLSASVGDRVTITCRTSENIYNNLAWYQQKPGKSPKLLIYAATNLADGVPSRFSGSGSGTDYTLTISSLQPEDFATYYCQHFWGTPLTFGGGTKVEIKRTVAAPSVFIFPPSDEQLKSGTASVVCLLNNFYPREAKVQWKVDNALQSGNSQESVTEQDSKDSTYSLSSTLTLSKADYEKHKVYACEVTHQGLSSPVTKSFNRGEC

SEQ ID NO: 64 - protein, 214 aa, synthetic construct
DIQMTQSPSSLSASVGDRVTITCRTSENIYNNLAWYQQKPGKAPKLLIYAATNLADGVPSRFSGSGSGTDYTLTISSLQPEDFATYYCQHFWGTPLTFGGGTKVEIKRTVAAPSVFIFPPSDEQLKSGTASVVCLLNNFYPREAKVQWKVDNALQSGNSQESVTEQDSKDSTYSLSSTLTLSKADYEKHKVYACEVTHQGLSSPVTKSFNRGEC

SEQ ID NO: 65 - protein, 214 aa, synthetic construct
DIQMTQSPSSLSASVGDRVTITCRTSENIYNNLAWYQQKPGKAPKLLIYAATNLAEGVPSRFSGSGSGTDYTLTISSLQPEDFATYYCQHFWGTPLTFGGGTKVEIKRTVAAPSVFIFPPSDEQLKSGTASVVCLLNNFYPREAKVQWKVDNALQSGNSQESVTEQDSKDSTYSLSSTLTLSKADYEKHKVYACEVTHQGLSSPVTKSFNRGEC

SEQ ID NO: 66 - protein, 214 aa, synthetic construct
DIQMTQSPSSLSASVGDRVTITCRTSENIYSNLAWYQQKPGKAPKLLIYAGTNLADGVPSRFSGSGSGTDYTLTISSLQPEDFANYYCQHFWGTPLTFGGGTKVEIKRTVAAPSVFIFPPSDEQLKSGTASVVCLLNNFYPREAKVQWKVDNALQSGNSQESVTEQDSKDSTYSLSSTLTLSKADYEKHKVYACEVTHQGLSSPVTKSFNRGEC

SEQ ID NO: 67-89 - skipped (23 entries)

SEQ ID NO: 90 - DNA, 20 bp, synthetic construct
  source 1..20: mol_type = other DNA
ctgtggaaagggtgaagcta

SEQ ID NO: 91 - DNA, 20 bp, synthetic construct
  source 1..20: mol_type = other DNA
gacaagggaactccaggatg

SEQ ID NO: 92 - DNA, 24 bp, synthetic construct
  source 1..24: mol_type = other DNA
agctctctcccagcttgatttcca

SEQ ID NO: 93 - DNA, 19 bp, synthetic construct
  source 1..19: mol_type = other DNA
aaggaccgacaagggaact

SEQ ID NO: 94 - DNA, 23 bp, synthetic construct
  source 1..23: mol_type = other DNA
ttctgacaacagtttgccgctgc

SEQ ID NO: 95 - DNA, 24 bp, synthetic construct
  source 1..24: mol_type = other DNA
gctgaattatttcttccgcagttg

SEQ ID NO: 96 - protein, 4 aa, synthetic construct
GGFG

SEQ ID NO: 97 - protein, 4 aa, synthetic construct
ALAL

SEQ ID NO: 98 - protein, 4 aa, synthetic construct
GFLG

SEQ ID NO: 99 - skipped

SEQ ID NO: 100 - DNA, 30 bp, synthetic construct
  source 1..30: mol_type = other DNA
cgccatttctcaacagatctgtcaaatcgc

SEQ ID NO: 101 - DNA, 30 bp, synthetic construct
  source 1..30: mol_type = other DNA
ccgccatttctcaacagatctgtcaaatcg

SEQ ID NO: 102 - DNA, 30 bp, synthetic construct
  source 1..30: mol_type = other DNA
gccgccatttctcaacagatctgtcaaatc

SEQ ID NO: 103 - DNA, 30 bp, synthetic construct
  source 1..30: mol_type = other DNA
agccgccatttctcaacagatctgtcaaat

SEQ ID NO: 104 - DNA, 30 bp, synthetic construct
  source 1..30: mol_type = other DNA
aagccgccatttctcaacagatctgtcaaa

SEQ ID NO: 105 - DNA, 30 bp, synthetic construct
  source 1..30: mol_type = other DNA
aaagccgccatttctcaacagatctgtcaa

SEQ ID NO: 106 - DNA, 30 bp, synthetic construct
  source 1..30: mol_type = other DNA
aaaagccgccatttctcaacagatctgtca

SEQ ID NO: 107 - DNA, 30 bp, synthetic construct
  source 1..30: mol_type = other DNA
aaaacgccgccatttctcaacagatctgtc

SEQ ID NO: 108 - DNA, 30 bp, synthetic construct
  source 1..30: mol_type = other DNA
gaaaacgccgccatttctcaacagatctgt

SEQ ID NO: 109 - DNA, 30 bp, synthetic construct
  source 1..30: mol_type = other DNA
tgaaaacgccgccatttctcaacagatctg

SEQ ID NO: 110 - DNA, 30 bp, synthetic construct
  source 1..30: mol_type = other DNA
atgaaaacgccgccatttctcaacagatct

SEQ ID NO: 111 - DNA, 30 bp, synthetic construct
  source 1..30: mol_type = other DNA
cataatgaaaacgccgccatttctcaacag

SEQ ID NO: 112 - DNA, 25 bp, synthetic construct
  source 1..25: mol_type = other DNA
catttctcaacagatctgtcaaatc

SEQ ID NO: 113 - DNA, 25 bp, synthetic construct
  source 1..25: mol_type = other DNA
gccatttctcaacagatctgtcaaa

SEQ ID NO: 114 - DNA, 25 bp, synthetic construct
  source 1..25: mol_type = other DNA
cgccatttctcaacagatctgtcaa

SEQ ID NO: 115 - DNA, 25 bp, synthetic construct
  source 1..25: mol_type = other DNA
gccgccatttctcaacagatctgtc

SEQ ID NO: 116 - DNA, 26 bp, synthetic construct
  source 1..26: mol_type = other DNA
cgccatttctcaacagatctgtcaaa

SEQ ID NO: 117 - DNA, 26 bp, synthetic construct
  source 1..26: mol_type = other DNA
ccgccatttctcaacagatctgtcaa

SEQ ID NO: 118 - DNA, 26 bp, synthetic construct
  source 1..26: mol_type = other DNA
cgccgccatttctcaacagatctgtc

SEQ ID NO: 119 - DNA, 26 bp, synthetic construct
  source 1..26: mol_type = other DNA
acgccgccatttctcaacagatctgt

SEQ ID NO: 120 - DNA, 27 bp, synthetic construct
  source 1..27: mol_type = other DNA
ccgccatttctcaacagatctgtcaaa

SEQ ID NO: 121 - DNA, 27 bp, synthetic construct
  source 1..27: mol_type = other DNA
gccgccatttctcaacagatctgtcaa

SEQ ID NO: 122 - DNA, 27 bp, synthetic construct
  source 1..27: mol_type = other DNA
cgccgccatttctcaacagatctgtca

SEQ ID NO: 123 - DNA, 27 bp, synthetic construct
  source 1..27: mol_type = other DNA
acgccgccatttctcaacagatctgtc

SEQ ID NO: 124 - DNA, 28 bp, synthetic construct
  source 1..28: mol_type = other DNA
cgccatttctcaacagatctgtcaaatc

SEQ ID NO: 125 - DNA, 28 bp, synthetic construct
  source 1..28: mol_type = other DNA
ccgccatttctcaacagatctgtcaaat

SEQ ID NO: 126 - DNA, 28 bp, synthetic construct
  source 1..28: mol_type = other DNA
gccgccatttctcaacagatctgtcaaa

SEQ ID NO: 127 - DNA, 28 bp, synthetic construct
  source 1..28: mol_type = other DNA
cgccgccatttctcaacagatctgtcaa

SEQ ID NO: 128 - DNA, 28 bp, synthetic construct
  source 1..28: mol_type = other DNA
acgccgccatttctcaacagatctgtca

SEQ ID NO: 129 - DNA, 28 bp, synthetic construct
  source 1..28: mol_type = other DNA
aacgccgccatttctcaacagatctgtc

SEQ ID NO: 130 - DNA, 28 bp, synthetic construct
  source 1..28: mol_type = other DNA
ctttatatcataatgaaaacgccgccat

SEQ ID NO: 131 - DNA, 28 bp, synthetic construct
  source 1..28: mol_type = other DNA
tctttatatcataatgaaaacgccgcca

SEQ ID NO: 132 - DNA, 28 bp, synthetic construct
  source 1..28: mol_type = other DNA
atctttatatcataatgaaaacgccgcc

SEQ ID NO: 133 - DNA, 25 bp, synthetic construct
  source 1..25: mol_type = other DNA
gccgccatttctcaacagatctgtc

SEQ ID NO: 134 - RNA, 148 nt, Homo sapiens
  source 1..148: mol_type = mRNA
gcgatttgacagatctgttgagaaatggcggcgttttcattatgatataaagatatttaatcagtggctaacagaagctgaacagtttctcagaaagacacaaattcctgagaattgggaacatgctaaatacaaatggtatcttaag